European Patent Application EP 4 632 062 A1, published October 15, 2025. Title: 락티플란티바실러스 플란타룸 균주, 그의 유래의 배양액 및 그의 항알러지 용도. Applicant: 지아이바이옴. The sequence listing filed with the application follows.

SEQUENCE LISTING (2 sequences)

SEQ ID NO: 1 - DNA, 1430 bp, synthetic construct
  source 1..1430: mol_type = other DNA
tcgaacgaactctggtattgattggtgcttgcatcatgatttacatttgagtgagtggcgaactggtgagtaacacgtgggaaacctgcccagaagcgggggataacacctggaaacagatgctaataccgcataacaacttggaccgcatggtccgagtttgaaagatggcttcggctatcacttttggatggtcccgcggcgtattagctagatggtgaggtaacggctcaccatggcaatgatacgtagccgacctgagagggtaatcggccacattgggactgagacacggcccaaactcctacgggaggcagcagtagggaatcttccacaatggacgaaagtctgatggagcaacgccgcgtgagtgaagaagggtttcggctcgtaaaactctgttgttaaagaagaacatatctgagagtaactgttcaggtattgacggtatttaaccagaaagccacggctaactacgtgccagcagccgcggtaatacgtaggtggcaagcgttgtccggatttattgggcgtaaagcgagcgcaggcggttttttaagtctgatgtgaaagccttcggctcaaccgaagaagtgcatcggaaactgggaaacttgagtgcagaagaggacagtggaactccatgtgtagcggtgaaatgcgtagatatatggaagaacaccagtggcgaaggcggctgtctggtctgtaactgacgctgaggctcgaaagtatgggtagcaaacaggattagataccctggtagtccataccgtaaacgatgaatgctaagtgttggagggtttccgcccttcagtgctgcagctaacgcattaagcattccgcctggggagtacggccgcaaggctgaaactcaaaggaattgacgggggcccgcacaagcggtggagcatgtggtttaattcgaagctacgcgaagaaccttaccaggtcttgacatactatgcaaatctaagagattagacgttcccttcggggacatggatacaggtggtgcatggttgtcgtcagctcgtgtcgtgagatgttgggttaagtcccgcaacgagcgcaacccttattatcagttgccagcattaagttgggcactctggtgagactgccggtgacaaaccggaggaaggtggggatgacgtcaaatcatcatgccccttatgacctgggctacacacgtgctacaatggatggtacaacgagttgcgaactcgcgagagtaagctaatctcttaaagccattctcagttcggattgtaggctgcaactcgcctacatgaagtcggaatcgctagtaatcgcggatcagcatgccgcggtgaatacgttcccgggccttgtacacaccgcccgtcacaccatgagagtttgtaacacccaaagtcggtggggtaaccttttaggaaccagccgcc

SEQ ID NO: 2 - DNA, 702 bp, synthetic construct
  source 1..702: mol_type = other DNA
atttcggtaaaggggcgattatgcggatgggtgacgctgcccagacgactatttcaacgatttcaagtggatcgttggccttagatgacgcgttgggtgtcggcggctacccacgtggtcggatcgtggaaatctacggtcctgaaagttcaggtaaaacgaccgtggcactacatgcggttgctgaagttcaaaagcagggtggtacggcggcctatatcgatgctgaaaacgcactagaccccgtttatgcggaacacctaggggtcaacattgatgacctgttactttcgcaaccagatactggtgaacaagggcttgaaattgcggatgccttagtttccagtggtgcggtcgatattttagttgttgactcggtggcggccttagtgccacgtgccgaaattgaaggtgaaatgggtgacgcacacgttgggttacaagcgcggctgatgtcacaagcgctccggaagttatcagggacattgaacaaaaccaagacaatcgcgttatttatcaatcaaattcgtgaaaaagttggtgtgatgtttggtaatcctgaaacgactcctggtggtcgggccttgaaattttacgccacgattcgtttggaagtacggcgggcagaacagatcaaggaaggaaccaatattattggtaaccgtgtccggatcaaagtcgttaagaacaaggttgcaccgc